European Patent Specification EP 4 232 092 B1, published May 27, 2026. Title: HYDROPHOBIC DRUGS IN ORGANIC CORE. Applicant: Northwestern University. Application Not Yet Assigned. The sequence listing filed with the application follows.

SEQUENCE LISTING (4 sequences)

SEQ ID NO: 1 - DNA, 9 bp, Artificial Sequence
  Synthetic
aggtcggct

SEQ ID NO: 2 - DNA, 18 bp, Artificial Sequence
  Synthetic
ttgttaatatgagtcgtt

SEQ ID NO: 3 - DNA, 9 bp, Artificial Sequence
  Synthetic
agccgacct

SEQ ID NO: 4 - DNA, 18 bp, Artificial Sequence
  Synthetic
aacgactcatattaacaa